European Patent Specification EP 3 639 849 B1, published July 30, 2025. Title: Vaccine. Applicant: The Pirbright Institute. The sequence listing filed with the application follows.

SEQUENCE LISTING (45 sequences)

SEQ ID NO: 1 - protein, 350 aa, African swine fever virus
MVLSLQTLTKKVLASQYPAKCHPHFLKCCGLWWHNGPIMYHQKKIWTPYFKNGTNLNAALVKAVEENNHDLIELFTEWGANINYGLLSVNTEHTRDLCRQLGAKEQLNDQEILRFFYTLKRDLTSSNIIFCHEVFSNNPILDTINRFEVKGMIYEQLEGLMVETDILSEMFTKYWYAMAIEFNLKEAICYFYQRYAHLHRWRLMCALFYNNVFDLHELYAKEKVRMDMDEMLRWACRKNYNYLTIYYCCVALGADINQAMFHSIQFYNIGNIFFCIDLGANAFEEGKTLAHQKDNSFIASMLSLNCYSMNDSLSLKETDPEVIKRMLKDYHSKNLSIAHKHYINDGFNDI

SEQ ID NO: 2 - protein, 356 aa, African swine fever virus
MVPSLQSFAKKVLASQHVSIDYHVILERCGLWWYKAPISLDCKHMLIKLPNFADGLDLNTALMLATKENNYQLIKMFTDWGADINYGLICANTPPIREFCWELGAKYQVDKKKIMHIFFKLIHPNTTSNNIILCLKFFNDNPFSAYVIIREIKSCIHWKLKNLAEDTNVLSNISDGDMLTIYCFIVALQDNLREAISYVYQHFKYLNTWWLTCALCYNKLFDLHNLYEKEKIRMDMDEMMRIACTKDNNFLTIYYCFILGANINLAMIASIRFYNMDNLFFCIDLGADAFEEAKALAEQQNYYLISHRLSLDIYSPDSSLLTLKEADPNKIYRLLKNYKSKSMLAYLNYDINDTSL

SEQ ID NO: 3 - protein, 353 aa, African swine fever virus
MLPSLQSLTKKVLAGQCVSVDHYHILKCCGLWWHNGPIMLHIRRNKLFIRSTCFSQGIELNIGLMKAVKENNHDLIKLFTEWGADINYGMICALTENTRDLCKELGAKEYLEREYILKIFFDTTRDKTSSNIIFCHEVFSNNPNLRIIDNLDLRGEIMWELRGLMEITFMLDHDDSFSTVLTKYWYAIAVDYDLKDAIRYFYQKYPRLHRWRLMCALFYNNVFDLHELYEIERVRMDIDEMMHIACIQDYSYSAIYYCFIMGANINQAMLVSIQNYNLGNLFFCIDLGANAFEEGKALAEQKENYLIAHALSLKHYNPVISLLSNVMDPEKINYMLKNYHSINMGIFLDYEQR

SEQ ID NO: 4 - protein, 350 aa, African swine fever virus
MLPSLQSLTKKVLAGQCVPTNQHYLLKYYDLWWYNAPITFDHNLRLIKSSGIKEGLDLNTALVKAVRENNYSLIKLFTEWGADINYGLVSVNTEHTRDLCQELGAKEILNEEEILQIFIDLKFHKTSSNIILCHEVFSNNPILQKVNNLKLRIEIFWELRELIEKTDLLNNEFLLSTLLLKYWYAIAVRYSLKEAIQYFYQKYTHMNTWRLTCALCFNNVFDLHEAYEKDKIHMDIEEMMRIACIKDHNLSTMYYCYMLGANINQAMLTSIQYYNIENMFFCMDLGADVFEEGTTALGEGYELIKNILSLKIYSPTTIPLPKSTDPEIIDHALKNYFSKNMMIFLSYDLR

SEQ ID NO: 5 - protein, 353 aa, African swine fever virus
MSLPLSLQTLVKKTVASQCLSIDEHCILKYCGLWWHDAPLKLCMDRGRIQIKSGFLGEDIDLRVALIIAVKENNYSLIKLFTEWGANINYSLLSINTKHIRELCRQLGAKETLEDNDIFRIFTRIMHNKTSGSIILCHEIFMNNPMLENKFVIQLRGLIYKRLWGLIEIKETDELNDLLVKYWYAKAVQYVCKNAICFLDEKYTDLNEWRLKCLLYYNKIYELHEMYHKKKVQIDVHDMICLACAKDNNLLTIYYCYALGGNINQAMLTSVQYYNVGNIFFCIDLGGNAFEEGRAIAEQKGYNFLSHSLTLDIYSSDASLPLNLKDPEKISSLLKDYKSKNLSIIWEYSHNIL

SEQ ID NO: 6 - protein, 357 aa, African swine fever virus
MLSLQTLAKKVVACNYLSSDYDYTLQRFGLWWDLGPIHLCNNCKQVFSYKHLQCFSEDDLCLEAALVKAVKSDNLELIRLFVDWGANPEYGLIRVPAVYLKRLCAELGGLTPVSEPRLLEILKEVANLKSCAGVLLGYDMFCHNPLLETVTRTTLDTVTYTCSNIPLTGDTAHLLLTKFWFALALRHNFTKAIHYFYKRHKNQLYWRVACSLYFNNIFDIHELCREKEICISPNLMMKFACLREKNYAAIYYCHRLGASLDYGMNLSIYNNNTLNMFFCIDLGAADFDRAQLIAHKAYMYNLSNIFLVKQLFSRDVTLVLDVTEPQEIYDMLKTYTSKNMKRAEEYLTAHPEIIVID

SEQ ID NO: 7 - protein, 531 aa, African swine fever virus
MFSLQNLCRKTLPDCKLPEFFDDYILQLLGLYWENHGTIQRAGNNCVLIQQHTLIPVNEALRIAASEENYEIVGLLLAWEGNLYYAIIGALEGNRYNLIRKYDDQIKDHHDILPFIDDPIIFHKCHIMRRCFFDCILYQAVKYSKFRVLLYFKYTLEDDLPLVHLLIEKACEDHNYEVIKWIYENLHVCHIIDTFDCAIAHKDLRLYCLGYTFIYNRIVPYKYHHLDILILSSLQLLHKVAAKGYLDFILETLKYDHNIDNLDVILTQAATYNHRKILTYFIPQSTYAQIEQCLFVAIKTKSSKKTLNLLLSHLNLSIKLIQKISQYVATFNSTNIIGILSMKRKKKIYLDIILTKFVKNAIFNKFVVRCMERFSINPERIVKMAARINKMMLVKKISEHVWKNHAARLKHLKHAVHTMKHKDGKNRLMNFIYEHCYYHMQGEEIFSLARFYAIHHAPKLFDVFYNCCILDTIRFKSLLLDCSHIIGKNAHDATNINIVNKYIGNLFAMGVLSKKEILQDYPSIYSKHYMP

SEQ ID NO: 8 - protein, 526 aa, African swine fever virus
MFSLQDLCRKHLFILPDVFGEHVLQRLGLYWRCHGSLQRIGDDHILIRRDLILSTNEALRMAGEEGNNEVVKLLLLWKGNLHYAVIGALQGDQYDLIHKYENQIGDFHFILPLIQDANTFEKCHALERFCGVSCLLKHATKYNMLPILQKYQEELSMRAYLHETLFELACLWQRYDVLKWIEQTMHVYDLKIMFNIAISKRDLTMYSLGYIFLFDRGNTEATLLTQHLEKTAAKGLLHFVLETLKYGGNIDTVLTQAVKYNHRKLLDYFLRQLPRKHIEKLLLLAVQEKASKKTLNLLLSHLNYSVKRIKKLLRYVIEYESTLVIKILLKKRVNLIDAMLEKMVRYFSATKVRTIMDELSISPERVIKMAIQKMRTDIVIHTSYVWEDDLERLTRLKNMVYTIKYEHGKKMLIKVMHGIYKNLLYGEREKVMFHLAKLYVAQNAATQFRDICKDCYKLDVARFKPRFKQLILDCLEIVTKKSCYSILEILEKHIISLFTMKVMTEEEKNLCLEILYKVIHYKTIQC

SEQ ID NO: 9 - protein, 280 aa, African swine fever virus
MSSSLQELCRKKLPDCILPEFFDDYVLQLLGLHWQDHGSLQRIEKNQILVQQEPIHINEALKVAASEGNYEIVELLLSWEADPRYAVVGALESKYYDLVYKYYDLVKDCHDILPLIQNPETFEKCHELNNPCSLKCLFKHAVIHDMLPILQKYTYFLDGWEYCNQMLFELACSKKKYEMVVWIEGVLGIGKVTSLFTIAISNRDLHLYSLGHLIILERMQSCGQDPTFLLNHFLRDVSIKGLLPFVLKTIEYGGSKEIAITLAKKYQHKHILKYFETGKC

SEQ ID NO: 10 - protein, 505 aa, African swine fever virus
MFSLQDICRKYLFQLPDSFDEYTLQVLGLYWEKHGSLQRIRKDAVFVQRNLIISINEALRIAASEGNGRVVKLLLSWEGNFHYVIIGALEGDHYDLIHKYGSQIEDYHMILSSIHNANTFEKCHELSNCDMWCLIQNAIKYNMLPILQKHRNILTHEGENQELFEMACEEQKYDIVLWIGQTLMLNEPEFIFDIAFERIDFSLLTMGYSLLFNNKMSSIDIHDEEDLISLLTEHLEKAATKGCFFFMLETLKHGGNVNMAVLSKAVEYNHRKILDYFIRQKCLSRKDIEKLLLVAISNSASKKTLNLLLSYLNHSVKNIIGKIVQSVLKNGDFTIIIFLKKKKINLVEPALIGFINYYYSYCFLEQFIHEFDIRPEKMIKMAARKGKLNMIIEFLNEKYVHKDDLGAIFKFLKNLVCTMKHKKGKETLIVLIHKIYQVIQLETKEKFKLLRFYVMHDATIQFISMYKDCFNLAGFKPFLLECLDIAIKKNYPDMIRNIETLLKCE

SEQ ID NO: 11 - protein, 254 aa, African swine fever virus
MQNKIPNFNLFFFFLYRMLEIVLATLLGDLQRLRVLTPQQRAVAFFRANTKELEDFLRSDGQSEEILSGPLLNRLLEPSCPLDILTGYHLFRQNPKAGQLRGLEVKMLERLYDANIYNILSRLRPKKVRNKAIELYWVFRAIHICHAPLVLDIVRYEEPDFAELAFICAAYFGEPQVMYLLYKYMPLTRAVLTDAIQISLESNNQVGICYAYLMGGSLKGLVSAPLRKRLRAKLRSQRKKKDVLSPHDFLLLLQ

SEQ ID NO: 12 - protein, 148 aa, African swine fever virus
MLERLYDANIYNILSRLRPEKVRNKAVELYWVFRAINMCHAPLVLDIVRYEEPDFAELAFICAAYFGEPQVMYLLYKYMPLTRAVLTDAIQISLESNSQVGICYAYLMGGSLKGLVRAPLRKRLRAKLRSQRKKKDVLPPHDFLLLLQ

SEQ ID NO: 13 - protein, 151 aa, African swine fever virus
MLERLYDANIYNMLARLRPELVRDKAIELYWLFRAILMCHSPLVLEIVRHETMDFAETAFICAAYFSEPQVMYALYKFIPISRAVLADAIQMCLESNSEAGICYAYLMGGSLKGKVPGSLRKRLRASPLRQERKKKNVLPPHEFLLMLHGI

SEQ ID NO: 14 - protein, 219 aa, African swine fever virus
MQRAVAFFRVNTKELEDFLYPDGQSEELLPGLLLNRLLEPSGPIDILTGYHLFRENPKAGRLRGLEVKLLERLYDANIYNMLAQIRPELVRIKAIELYWLFRAILMCHSPLVLEIVRHETMDFAELAFICAAYFSEPQVMYALYKFIPISRAVLADAIEMSLESNSETGICYAYLMGGSLKGKVPGPLRKRLRASPLRQERKKKNVLPPHEFLLMLHGI

SEQ ID NO: 15 - protein, 254 aa, African swine fever virus
MQNKIPNFNLFFFFLYRMLEIVLATLLGDLQRLRVLTPQQRAVAFFRANTKELEDFLCSDGQSEEILSGPLLNRLLEPSGPLDILTGYHLFRQNPKAGQLRGLEVKMLERLYDANIYNILSRLRPEKVRNKAIELYWVFRAIHICHAPLVLDIVRYEEPDFAELAFICAAYFGEPQVMYLLYKYMPLTRAVLTDAIRISLESNNQVGICYAYLMGGSLKGLVSAPLRKRLCAKLRSQRKKKDVLSPHDFLLLLQ

SEQ ID NO: 16 - protein, 148 aa, African swine fever virus
MLERLYDANIYNILSRLRPEKVRNKAVELYWVFRAINMCHAPLVLDIVRYEEPDFAELAFICAAYFGEPQVMYLLYKYMPLSRAVLTDAIQISLESNSQVGICYAYLMGGSLKGLVRAPLRKRLRAKLRSQRKKKDVLPPHDFLLLLQ

SEQ ID NO: 17 - protein, 148 aa, African swine fever virus
MLERLYDANIYNILSRLRPEKVRNKAVELYWVFRAINMCHAPLVLDIVRNEELDFAELAFICAAYFGEPQVMYLLYKYMPLTRAVLTDAIQISLESNSQVGICYAYLMGGSLKGLVRAPLRKRLRAKLRSQRKKKDVLPPHDFLLLLQ

SEQ ID NO: 18 - protein, 148 aa, African swine fever virus
MLERLYDANIYNILSRLRPEKVRNKAIELYWVFRAIHICHAPLVLDIVRYEEPDFAELAFICAAYFGEPQVMYLLYKYMPLTRAVLTDAIRISLESNNQVGICYAYLMGGSLKGLVSAPLRKRLRAKLRSQRKKKDVLSPHDFLLLLQ

SEQ ID NO: 19 - protein, 148 aa, African swine fever virus
MLERLYDANIYNILSRLRPEKVRNKAIELYWVFRAIHICHAPLVLDIVRYEEPDFAELAFICAAYFGEPQVMYLLYKYMPLTRAVLTDAIQISLESNNQVGICYAYLMGGSLKGLVSAPLRKRLRAKLRSQRKKKDVLSPHDFLLLLQ

SEQ ID NO: 20 - DNA, 36 bp, Artificial Sequence
  Primer FlankLF
acgttgcaaagcttccattaatccctccagttgttc

SEQ ID NO: 21 - DNA, 36 bp, Artificial Sequence
  Primer Flank LR
acgttgcaggtacccctctctctgcagactctcacc

SEQ ID NO: 22 - DNA, 36 bp, Artificial Sequence
  Primer Flank RF
acgttgcagcggccgcctctccaagacatctgtcgg

SEQ ID NO: 23 - DNA, 40 bp, Artificial Sequence
  Primer Flank RR
acgtacgtctcgagcctcacatgccatctcaaacaattcc

SEQ ID NO: 24 - DNA, 22 bp, Artificial Sequence
  Primer BeninD8F
ggtgagagtctgcagagagagg

SEQ ID NO: 25 - DNA, 18 bp, Artificial Sequence
  Primer BeninD8R
gccctagcacttgtaacg

SEQ ID NO: 26 - DNA, 27 bp, Artificial Sequence
  Primer RGUS
ccttctctgccgtttccaaatcgccgc

SEQ ID NO: 27 - DNA, 18 bp, Artificial Sequence
  Primer BeninD8INTF
cgatgtatcattgatgtc

SEQ ID NO: 28 - DNA, 19 bp, Artificial Sequence
  Primer BeninD8INTR
ggataatcttagggaggcc

SEQ ID NO: 29 - DNA, 19 bp, Artificial Sequence
  Primer 9LF
atgacgcattaaaccggcg

SEQ ID NO: 30 - DNA, 20 bp, Artificial Sequence
  Primer 4RR
cagtatagccctagcacttg

SEQ ID NO: 31 - DNA, 96 bp, Artificial Sequence
  Recombinant virus sequence (left flank of deletion/insertion)
agagaggggtaccatttaataaaaacaataaattattttttataacattatatataactttgtatagcatacattatacgaagttatatgttacgt

SEQ ID NO: 32 - DNA, 96 bp, African swine fever virus
agagaggaccatatttctttttttgaaaaaatcaaattaaaaaaaaacatgcttgtttggcatacatgtaactatgttataaccatgttataacca

SEQ ID NO: 33 - DNA, 73 bp, Artificial Sequence
  Recombinant virus sequence (right flank of deletion/insertion)
cagccagggaggcaaacaatgaggaattctgcagatatccatcactggcggccgcctctccaagacatcttgt

SEQ ID NO: 34 - DNA, 77 bp, African swine fever virus
ttttatcatacattaaaattccagtaaaatttatattttttttggtaaacaaatgttttctctccaagacatcttgt

SEQ ID NO: 35 - DNA, 2160 bp, African swine fever virus
aaatgaatagatttaatccaagtagtattaaaattttttagaaatagtgttctacaaataatgaaatgaatagcccaaaaaaaataaggtgtacattaatgtaatatattgttaggctaagtaaatttaatatttaaagtacttggaaaaatattttttaacatatgctgtctaggaatttttttagacatttaaaaccatatagttactttatttattacacttaacttgaaaagaattattgcctaaaatattaatagatgaagtaatattgtgtaattgagtccataacatgggtgggaaacaaaaatctcgtaatatgaaaaataaacatcctaaaaagagtgcaattgttataagtttatgtaactttattttaaagtaagaatataaaaatatgagtacaagaggaataggggccattactaatattggctccaacatcctgttgtctacaaaaaaaaatatttttttggcaaaaaaaaatccatggaaggatattaatacacataattgtttgacatcatattggtatacttaccaaatagtaatatacaaccatcctaatattcactttatgaaatgacccccccccccacctatacagtaaaatagtataggttttaataaagaaaaaagatattatgtagtttttatttttgtatagtgcgtgaatgcaaaataaaatcccaaattttaaccttttctttttttttctatacaggatgttagaaatagtattggcaacgctgctaggcgacctgcagcggctccgggttcttacccctcagcagcgggcggttgccttctttcgagccaatactaaggagctagaggacttcttacgctcagatgggcaatctgaggagatactgtctggccccctccttaaccgtctactagaaccctcatgccctcttgatattttaaccggatatcacctatttcgtcagaatcccaaggcaggtcagttgcgcggccttgaggtcaagatgcttgaacggttatacgatgctaatatttacaatatattgtctcggctgcgacctaaaaaagtccgcaacaaggctattgagctatactgggttttccgagctatccatatttgtcatgctcctttagttttagatattgtacgatatgaggaaccggactttgctgaactggcctttatttgtgctgcttactttggtgaacctcaggtaatgtatttgctctacaaatatatgcctctgacccgcgcagttcttacggatgccatccagataagtcttgagagcaacaaccaggtagggatttgctatgcttacttgatgggaggcagcctcaagggactagtctccgccccactgcgtaaacgtctgcgcgccaaactacgctcgcagcgcaaaaagaaggacgttctttcaccccacgacttcttactgctgctccagtagctttttttgccgcaggagcaccgtggataggagctcctccacgctcgcgatccggcgctggaagcggaaccgatcgaccgccacctgctcccagggacccttgcgctcgatgtcgtcggcttcccatacctcgacggctgcagcaaagcggacgtgcttcgtgtcattcgtccgttttttgcgccgccgccccccccccattattcctgtaagattagtgtttaatacctataataacataattttaagatttaatataccaaaacttaaactatttttgtatagtaactattagcatgtctacacatgattgtttttcaaaagagaaaccagttgatatgaacgatatatctgagaaatcatctgtcgtggataatgcacccgagaaaccagctggagcgaatcatatacctgagaagtcggcccgcgaaatgacatcatcagaatggattgctgaatattggaaaggtataaaacgtggaaatgacgtgccatgttgttgtccaagaaaaatgaccagtgcagacaaaaagttttcagtatttggtaagggatccctaatacgctccatccagaagaataattaaaaaaaatattttttttggtaagtttataaactatatagttaaatatggtaaaaaaaatcacataataattaaactgaacgtgttagaattaatatttttttataatcggatataatatccattaaatcaataaa

SEQ ID NO: 36 - DNA, 38 bp, Artificial Sequence
  Primer 360-18RFlankL-for-Benin
gctatccaagcttctacaaataatgaaatgaatagccc

SEQ ID NO: 37 - DNA, 38 bp, Artificial Sequence
  Primer 360-18RFlankL-rev-Benin2
gctatccggtacccataaagtgaatattaggatggttg

SEQ ID NO: 38 - DNA, 37 bp, Artificial Sequence
  Primer 360-18RFlankR-for
gctatccgcggccgccgacttcttactgctgctccag

SEQ ID NO: 39 - DNA, 36 bp, Artificial Sequence
  Primer 360-18RFlankR-rev
gctatcctctagatcttctggatggagcgtattagg

SEQ ID NO: 40 - DNA, 22 bp, Artificial Sequence
  Primer 18R-Benin-Pair1-For
gagtacaagaggaataggggcc

SEQ ID NO: 41 - DNA, 23 bp, Artificial Sequence
  Primer 18R-OURT-Pair1-Rev
gcatgacaaatatggatagctcg

SEQ ID NO: 42 - DNA, 21 bp, Artificial Sequence
  Primer 18R-OURT-Pair2-For
gtccgcaacaaggctattgag

SEQ ID NO: 43 - DNA, 19 bp, Artificial Sequence
  Primer 18R-OURT-Pair2-Rev
gacgtttacgcagtggggc

SEQ ID NO: 44 - DNA, 24 bp, Artificial Sequence
  Primer 18R-OURT-Pair3-For
caaccaggtagggatttgctatgc

SEQ ID NO: 45 - DNA, 16 bp, Artificial Sequence
  Primer 18R-OURT-Pair3-Rev
gctgcagccgtcgagg